European Patent Specification EP 3 443 010 B1, published August 7, 2024. Title: NEW ANTI-SIRPa ANTIBODIES AND THEIR THERAPEUTIC APPLICATIONS. Applicant: OSE IMMUNOTHERAPEUTICS. The sequence listing filed with the application follows.

SEQUENCE LISTING (73 sequences)

SEQ ID NO: 1 - protein, 7 aa, Homo sapiens
SLIPVGP

SEQ ID NO: 2 - protein, 12 aa, Homo sapiens
  MISC_FEATURE (1)..(1): Xaa = G or A
XRELIYNQKEGH

SEQ ID NO: 3 - protein, 10 aa, Homo sapiens
  MISC_FEATURE: Xaa = DV or T
  misc_feature (9)..(9): Xaa can be any naturally occurring amino acid
KFRKGSPDXE

SEQ ID NO: 4 - protein, 23 aa, Homo sapiens
QHTVSFTCESHGFSPRDITLKWF

SEQ ID NO: 5 - protein, 11 aa, Homo sapiens
ICEVAHVTLQG

SEQ ID NO: 6 - protein, 11 aa, Homo sapiens
YPQRLQLTWLE

SEQ ID NO: 7 - protein, 12 aa, Homo sapiens
GRELIYNQKEGH

SEQ ID NO: 8 - protein, 11 aa, Homo sapiens
KFRKGSPDDVE

SEQ ID NO: 9 - protein, 12 aa, Homo sapiens
ARELIYNQKEGH

SEQ ID NO: 10 - protein, 10 aa, Homo sapiens
KFRKGSPDTE

SEQ ID NO: 11 - protein, 7 aa, Homo sapiens
GRELIYN

SEQ ID NO: 12 - protein, 22 aa, Homo sapiens
HTVSFTCESHGFSPRDITLKWF

SEQ ID NO: 13 - protein, 7 aa, Homo sapiens
ARELIYN

SEQ ID NO: 14 - protein, 5 aa, Artificial Sequence
  Heavy chain CDR1
SYWVH

SEQ ID NO: 15 - protein, 17 aa, Artificial Sequence
  Heavy chain CDR2
NIDPSDSDTHYNQKFKD

SEQ ID NO: 16 - protein, 17 aa, Artificial Sequence
  Heavy chain CDR2
NIDPSDSDTHYSPSFQG

SEQ ID NO: 17 - protein, 11 aa, Artificial Sequence
  Heavy chain CDR3
GGTGTMAWFAY

SEQ ID NO: 18 - protein, 11 aa, Artificial Sequence
  Heavy chain CDR3
GGTGTLAWFAY

SEQ ID NO: 19 - protein, 11 aa, Artificial Sequence
  Heavy chain CDR3
GGTGTMAYFAY

SEQ ID NO: 20 - protein, 11 aa, Artificial Sequence
  Heavy chain CDR3
GGTGTLAYFAY

SEQ ID NO: 21 - protein, 16 aa, Artificial Sequence
  Light chain CDR1
RSSQSLVHSYGNTYLY

SEQ ID NO: 22 - protein, 7 aa, Artificial Sequence
  Light chain CDR2
RVSNRFS

SEQ ID NO: 23 - protein, 9 aa, Artificial Sequence
  Light chain CDR3
FQGTHVPYT

SEQ ID NO: 24 - protein, 120 aa, Artificial Sequence
  Heavy chain variable domain
QVQLQQPGAELVRPGSSVKLSCKASGYTFTSYWVHWVKQRPIQGLEWIGNIDPSDSDTHYNQKFKDKASLTVDKSSSTAYMQLSSLTFEDSAVYYCVRGGTGTMAWFAYWGQGTLVTVSA

SEQ ID NO: 25 - protein, 120 aa, Artificial Sequence
  Heavy chain variable domain
EVQLVQSGAEVKKPGESLRISCKASGYTFTSYWVHWVRQMPGKGLEWIGNIDPSDSDTHYNQKFKDHVTLSVDKSISTAYLQLSSLKASDTAMYYCVRGGTGTMAWFAYWGQGTLVTVSS

SEQ ID NO: 26 - protein, 120 aa, Artificial Sequence
  Heavy chain variable domain
EVQLVQSGAEVKKPGESLRISCKASGYSFTSYWVHWVRQMPGKGLEWMGNIDPSDSDTHYNQKFKDHVTLSVDKSISTAYLQLSSLKASDTAMYYCVRGGTGTMAWFAYWGQGTLVTVSS

SEQ ID NO: 27 - protein, 120 aa, Artificial Sequence
  Heavy chain variable domain
EVQLVQSGAEVKKPGESLRISCKASGYSFTSYWVHWVRQMPGKGLEWMGNIDPSDSDTHYSPSFQGHVTLSVDKSISTAYLQLSSLKASDTAMYYCVRGGTGTMAWFAYWGQGTLVTVSS

SEQ ID NO: 28 - protein, 120 aa, Artificial Sequence
  Heavy chain variable domain
EVQLVQSGAEVKKPGESLRISCKASGYSFTSYWVHWVRQMPGKGLEWMGNIDPSDSDTHYSPSFQGHVTLSVDKSISTAYLQLSSLKASDTAMYYCVRGGTGTLAWFAYWGQGTLVTVSS

SEQ ID NO: 29 - protein, 120 aa, Artificial Sequence
  Heavy chain variable domain
EVQLVQSGAEVKKPGESLRISCKASGYSFTSYWVHWVRQMPGKGLEWMGNIDPSDSDTHYSPSFQGHVTLSVDKSISTAYLQLSSLKASDTAMYYCVRGGTGTMAYFAYWGQGTLVTVSS

SEQ ID NO: 30 - protein, 120 aa, Artificial Sequence
  Heavy chain variable domain
EVQLVQSGAEVKKPGESLRISCKASGYSFTSYWVHWVRQMPGKGLEWMGNIDPSDSDTHYSPSFQGHVTLSVDKSISTAYLQLSSLKASDTAMYYCVRGGTGTLAYFAYWGQGTLVTVSS

SEQ ID NO: 31 - protein, 112 aa, Artificial Sequence
  Light chain variable domain
DVVMTQTPLSLPVSLGDQASISCRSSQSLVHSYGNTYLYWYLQKPGQSPKLLIYRVSNRFSGVPDRFSGSGSGTDFTLKISRVEAEDLGVYFCFQGTHVPYTFGSGTKLEIK

SEQ ID NO: 32 - protein, 112 aa, Artificial Sequence
  Light chain variable domain
DVVMTQSPLSLPVTLGQPASISCRSSQSLVHSYGNTYLYWYQQRPGQSPRLLIYRVSNRFSGVPDRFSGSGSGTDFTLKISRVEAEDVGVYFCFQGTHVPYTFGGGTKVEIK

SEQ ID NO: 33 - protein, 112 aa, Artificial Sequence
  Light chain variable domain
DVVMTQSPLSLPVTLGQPASISCRSSQSLVHSYGNTYLYWFQQRPGQSPRLLIYRVSNRFSGVPDRFSGSGSGTDFTLKISRVEAEDVGVYYCFQGTHVPYTFGGGTKVEIK

SEQ ID NO: 34 - protein, 327 aa, Artificial Sequence
  Heavy chain constant domain-IgG4m-S228P
ASTKGPSVFPLAPCSRSTSESTAALGCLVKDYFPEPVTVSWNSGALTSGVHTFPAVLQSSGLYSLSSVVTVPSSSLGTKTYTCNVDHKPSNTKVDKRVESKYGPPCPPCPAPEFLGGPSVFLFPPKPKDTLMISRTPEVTCVVVDVSQEDPEVQFNWYVDGVEVHNAKTKPREEQFNSTYRVVSVLTVLHQDWLNGKEYKCKVSNKGLPSSIEKTISKAKGQPREPQVYTLPPSQEEMTKNQVSLTCLVKGFYPSDIAVEWESNGQPENNYKTTPPVLDSDGSFFLYSRLTVDKSRWQEGNVFSCSVMHEALHNHYTQKSLSLSPGK

SEQ ID NO: 35 - protein, 107 aa, Artificial Sequence [sequence omitted]

SEQ ID NO: 36 - protein, 447 aa, Artificial Sequence
  Heavy chain sequence 18D5
QVQLQQPGAELVRPGSSVKLSCKASGYTFTSYWVHWVKQRPIQGLEWIGNIDPSDSDTHYNQKFKDKASLTVDKSSSTAYMQLSSLTFEDSAVYYCVRGGTGTMAWFAYWGQGTLVTVSAASTKGPSVFPLAPCSRSTSESTAALGCLVKDYFPEPVTVSWNSGALTSGVHTFPAVLQSSGLYSLSSVVTVPSSSLGTKTYTCNVDHKPSNTKVDKRVESKYGPPCPPCPAPEFLGGPSVFLFPPKPKDTLMISRTPEVTCVVVDVSQEDPEVQFNWYVDGVEVHNAKTKPREEQFNSTYRVVSVLTVLHQDWLNGKEYKCKVSNKGLPSSIEKTISKAKGQPREPQVYTLPPSQEEMTKNQVSLTCLVKGFYPSDIAVEWESNGQPENNYKTTPPVLDSDGSFFLYSRLTVDKSRWQEGNVFSCSVMHEALHNHYTQKSLSLSPGK

SEQ ID NO: 37 - protein, 447 aa, Artificial Sequence
  Heavy chain sequence HA
EVQLVQSGAEVKKPGESLRISCKASGYTFTSYWVHWVRQMPGKGLEWIGNIDPSDSDTHYNQKFKDHVTLSVDKSISTAYLQLSSLKASDTAMYYCVRGGTGTMAWFAYWGQGTLVTVSSASTKGPSVFPLAPCSRSTSESTAALGCLVKDYFPEPVTVSWNSGALTSGVHTFPAVLQSSGLYSLSSVVTVPSSSLGTKTYTCNVDHKPSNTKVDKRVESKYGPPCPPCPAPEFLGGPSVFLFPPKPKDTLMISRTPEVTCVVVDVSQEDPEVQFNWYVDGVEVHNAKTKPREEQFNSTYRVVSVLTVLHQDWLNGKEYKCKVSNKGLPSSIEKTISKAKGQPREPQVYTLPPSQEEMTKNQVSLTCLVKGFYPSDIAVEWESNGQPENNYKTTPPVLDSDGSFFLYSRLTVDKSRWQEGNVFSCSVMHEALHNHYTQKSLSLSPGK

SEQ ID NO: 38 - protein, 447 aa, Artificial Sequence
  Heavy chain sequence HB
EVQLVQSGAEVKKPGESLRISCKASGYSFTSYWVHWVRQMPGKGLEWMGNIDPSDSDTHYNQKFKDHVTLSVDKSISTAYLQLSSLKASDTAMYYCVRGGTGTMAWFAYWGQGTLVTVSSASTKGPSVFPLAPCSRSTSESTAALGCLVKDYFPEPVTVSWNSGALTSGVHTFPAVLQSSGLYSLSSVVTVPSSSLGTKTYTCNVDHKPSNTKVDKRVESKYGPPCPPCPAPEFLGGPSVFLFPPKPKDTLMISRTPEVTCVVVDVSQEDPEVQFNWYVDGVEVHNAKTKPREEQFNSTYRVVSVLTVLHQDWLNGKEYKCKVSNKGLPSSIEKTISKAKGQPREPQVYTLPPSQEEMTKNQVSLTCLVKGFYPSDIAVEWESNGQPENNYKTTPPVLDSDGSFFLYSRLTVDKSRWQEGNVFSCSVMHEALHNHYTQKSLSLSPGK

SEQ ID NO: 39 - protein, 447 aa, Artificial Sequence
  Heavy chain sequence HC
EVQLVQSGAEVKKPGESLRISCKASGYSFTSYWVHWVRQMPGKGLEWMGNIDPSDSDTHYSPSFQGHVTLSVDKSISTAYLQLSSLKASDTAMYYCVRGGTGTMAWFAYWGQGTLVTVSSASTKGPSVFPLAPCSRSTSESTAALGCLVKDYFPEPVTVSWNSGALTSGVHTFPAVLQSSGLYSLSSVVTVPSSSLGTKTYTCNVDHKPSNTKVDKRVESKYGPPCPPCPAPEFLGGPSVFLFPPKPKDTLMISRTPEVTCVVVDVSQEDPEVQFNWYVDGVEVHNAKTKPREEQFNSTYRVVSVLTVLHQDWLNGKEYKCKVSNKGLPSSIEKTISKAKGQPREPQVYTLPPSQEEMTKNQVSLTCLVKGFYPSDIAVEWESNGQPENNYKTTPPVLDSDGSFFLYSRLTVDKSRWQEGNVFSCSVMHEALHNHYTQKSLSLSPGK

SEQ ID NO: 40 - protein, 447 aa, Artificial Sequence
  Heavy chain sequence HE
EVQLVQSGAEVKKPGESLRISCKASGYSFTSYWVHWVRQMPGKGLEWMGNIDPSDSDTHYSPSFQGHVTLSVDKSISTAYLQLSSLKASDTAMYYCVRGGTGTLAWFAYWGQGTLVTVSSASTKGPSVFPLAPCSRSTSESTAALGCLVKDYFPEPVTVSWNSGALTSGVHTFPAVLQSSGLYSLSSVVTVPSSSLGTKTYTCNVDHKPSNTKVDKRVESKYGPPCPPCPAPEFLGGPSVFLFPPKPKDTLMISRTPEVTCVVVDVSQEDPEVQFNWYVDGVEVHNAKTKPREEQFNSTYRVVSVLTVLHQDWLNGKEYKCKVSNKGLPSSIEKTISKAKGQPREPQVYTLPPSQEEMTKNQVSLTCLVKGFYPSDIAVEWESNGQPENNYKTTPPVLDSDGSFFLYSRLTVDKSRWQEGNVFSCSVMHEALHNHYTQKSLSLSPGK

SEQ ID NO: 41 - protein, 447 aa, Artificial Sequence
  Heavy chain sequence HF
EVQLVQSGAEVKKPGESLRISCKASGYSFTSYWVHWVRQMPGKGLEWMGNIDPSDSDTHYSPSFQGHVTLSVDKSISTAYLQLSSLKASDTAMYYCVRGGTGTMAYFAYWGQGTLVTVSSASTKGPSVFPLAPCSRSTSESTAALGCLVKDYFPEPVTVSWNSGALTSGVHTFPAVLQSSGLYSLSSVVTVPSSSLGTKTYTCNVDHKPSNTKVDKRVESKYGPPCPPCPAPEFLGGPSVFLFPPKPKDTLMISRTPEVTCVVVDVSQEDPEVQFNWYVDGVEVHNAKTKPREEQFNSTYRVVSVLTVLHQDWLNGKEYKCKVSNKGLPSSIEKTISKAKGQPREPQVYTLPPSQEEMTKNQVSLTCLVKGFYPSDIAVEWESNGQPENNYKTTPPVLDSDGSFFLYSRLTVDKSRWQEGNVFSCSVMHEALHNHYTQKSLSLSPGK

SEQ ID NO: 42 - protein, 447 aa, Artificial Sequence
  Heavy chain sequence HEF
EVQLVQSGAEVKKPGESLRISCKASGYSFTSYWVHWVRQMPGKGLEWMGNIDPSDSDTHYSPSFQGHVTLSVDKSISTAYLQLSSLKASDTAMYYCVRGGTGTLAYFAYWGQGTLVTVSSASTKGPSVFPLAPCSRSTSESTAALGCLVKDYFPEPVTVSWNSGALTSGVHTFPAVLQSSGLYSLSSVVTVPSSSLGTKTYTCNVDHKPSNTKVDKRVESKYGPPCPPCPAPEFLGGPSVFLFPPKPKDTLMISRTPEVTCVVVDVSQEDPEVQFNWYVDGVEVHNAKTKPREEQFNSTYRVVSVLTVLHQDWLNGKEYKCKVSNKGLPSSIEKTISKAKGQPREPQVYTLPPSQEEMTKNQVSLTCLVKGFYPSDIAVEWESNGQPENNYKTTPPVLDSDGSFFLYSRLTVDKSRWQEGNVFSCSVMHEALHNHYTQKSLSLSPGK

SEQ ID NO: 43 - protein, 219 aa, Artificial Sequence
  Light chain sequence 18D5
DVVMTQTPLSLPVSLGDQASISCRSSQSLVHSYGNTYLYWYLQKPGQSPKLLIYRVSNRFSGVPDRFSGSGSGTDFTLKISRVEAEDLGVYFCFQGTHVPYTFGSGTKLEIKRTVAAPSVFIFPPSDEQLKSGTASVVCLLNNFYPREAKVQWKVDNALQSGNSQESVTEQDSKDSTYSLSSTLTLSKADYEKHKVYACEVTHQGLSSPVTKSFNRGEC

SEQ ID NO: 44 - protein, 219 aa, Artificial Sequence
  Light chain sequence LA
DVVMTQSPLSLPVTLGQPASISCRSSQSLVHSYGNTYLYWYQQRPGQSPRLLIYRVSNRFSGVPDRFSGSGSGTDFTLKISRVEAEDVGVYFCFQGTHVPYTFGGGTKVEIKRTVAAPSVFIFPPSDEQLKSGTASVVCLLNNFYPREAKVQWKVDNALQSGNSQESVTEQDSKDSTYSLSSTLTLSKADYEKHKVYACEVTHQGLSSPVTKSFNRGEC

SEQ ID NO: 45 - protein, 219 aa, Artificial Sequence
  Light chain sequence LB
DVVMTQSPLSLPVTLGQPASISCRSSQSLVHSYGNTYLYWFQQRPGQSPRLLIYRVSNRFSGVPDRFSGSGSGTDFTLKISRVEAEDVGVYYCFQGTHVPYTFGGGTKVEIKRTVAAPSVFIFPPSDEQLKSGTASVVCLLNNFYPREAKVQWKVDNALQSGNSQESVTEQDSKDSTYSLSSTLTLSKADYEKHKVYACEVTHQGLSSPVTKSFNRGEC

SEQ ID NO: 46 - DNA, 360 bp, Artificial Sequence
  Nucleic acid sequence coding the heavy chain variable domain 18D5
caggtgcagctgcagcagccaggagctgagctggtgaggcctggctccagcgtgaagctgtcctgcaaggctagcggctacaccttcacaagctattgggtgcactgggtgaagcagcggccaatccagggcctggagtggatcggcaacatcgaccccagcgactctgatacccattacaatcagaagtttaaggacaaggcctctctgaccgtggataagtcttccagcacagcttatatgcagctgtcttccctgacattcgaggattccgccgtgtactattgcgtgaggggaggaaccggaacaatggcttggtttgcttactggggccagggcaccctggtgacagtgtctgct

SEQ ID NO: 47 - DNA, 360 bp, Artificial Sequence
  Nucleic acid sequence coding the heavy chain variable domain HA
gaggtgcagctggtgcagagcggagctgaggtgaagaagccaggcgagtctctgaggatctcctgcaaggctagcggctacaccttcacatcttattgggtgcactgggtgcggcagatgccaggcaagggcctggagtggatcggcaacatcgaccctagcgactctgatacccactacaatcagaagtttaaggaccatgtgaccctgtctgtggataagtccatcagcacagcctatctgcagctgtccagcctgaaggcctccgatacagctatgtactattgcgtgaggggaggaaccggaacaatggcttggttcgcttactggggccagggcaccctggtgacagtgtcttcc

SEQ ID NO: 48 - DNA, 360 bp, Artificial Sequence
  Nucleic acid sequence coding the heavy chain variable domain HB
gaggtgcagctggtgcagtccggagctgaggtgaagaagccaggcgagtctctgaggatctcctgcaaggcttctggctactccttcaccagctattgggtgcactgggtgcggcagatgccaggcaagggcctggagtggatgggcaacatcgaccctagcgactctgatacacactacaatcagaagtttaaggaccatgtgaccctgagcgtggataagtccatcagcacagcctatctgcagctgtccagcctgaaggcctctgataccgctatgtactattgcgtgaggggaggaaccggaacaatggcttggttcgcttactggggccagggcaccctggtgacagtgtcttcc

SEQ ID NO: 49 - DNA, 360 bp, Artificial Sequence
  Nucleic acid sequence coding the heavy chain variable domain HC
gaggtgcagctggtgcagtctggcgccgaggtgaagaagccaggcgagagcctgaggatctcttgcaaggctagcggctactctttcacctcctattgggtgcactgggtgcggcagatgccaggcaagggcctggagtggatgggcaacatcgaccccagcgactctgatacacactactcccctagctttcagggccatgtgaccctgtccgtggacaagtctatctccacagcctatctgcagctgtccagcctgaaggccagcgataccgctatgtactattgcgtgaggggaggaaccggaacaatggcttggttcgcttactggggccagggcaccctggtgacagtgtcttcc

SEQ ID NO: 50 - DNA, 360 bp, Artificial Sequence
  Nucleic acid sequence coding the heavy chain variable domain HE
gaggtgcagctggtgcagtctggcgccgaggtgaagaagccaggcgagagcctgaggatctcttgcaaggctagcggctactctttcacctcctattgggtgcactgggtgcggcagatgccaggcaagggcctggagtggatgggcaacatcgaccccagcgactctgatacacactactcccctagctttcagggccatgtgaccctgtccgtggacaagtctatctccacagcctatctgcagctgtccagcctgaaggccagcgataccgctatgtactattgcgtgaggggaggaaccggcacactggcttggttcgcttactggggccagggcaccctggtgacagtgtcttcc

SEQ ID NO: 51 - DNA, 360 bp, Artificial Sequence
  Nucleic acid sequence coding the heavy chain variable domain HF
gaggtgcagctggtgcagtctggcgccgaggtgaagaagccaggcgagagcctgaggatctcttgcaaggctagcggctactctttcacctcctattgggtgcactgggtgcggcagatgccaggcaagggcctggagtggatgggcaacatcgaccccagcgactctgatacacactactcccctagctttcagggccatgtgaccctgtccgtggacaagtctatctccacagcctatctgcagctgtccagcctgaaggccagcgataccgctatgtactattgcgtgaggggaggaaccggaacaatggcttacttcgcttattggggccagggcaccctggtgacagtgtcttcc

SEQ ID NO: 52 - DNA, 360 bp, Artificial Sequence
  Nucleic acid sequence coding the heavy chain variable domain HEF
gaggtgcagctggtgcagtctggcgccgaggtgaagaagccaggcgagagcctgaggatctcttgcaaggctagcggctactctttcacctcctattgggtgcactgggtgcggcagatgccaggcaagggcctggagtggatgggcaacatcgaccccagcgactctgatacacactactcccctagctttcagggccatgtgaccctgtccgtggacaagtctatctccacagcctatctgcagctgtccagcctgaaggccagcgataccgctatgtactattgcgtgaggggaggaaccggcacactggcttacttcgcttattggggccagggcaccctggtgacagtgtcttcc

SEQ ID NO: 53 - DNA, 336 bp, Artificial Sequence
  Nucleic acid sequence coding the light chain variable domain 18D5
gacgtggtcatgacccagacaccactgagcctgcccgtgtccctgggcgatcaggcctctatctcctgcaggtccagccagtccctggtgcacagctatggcaacacatacctgtattggtacctgcagaagccaggccagtcccccaagctgctgatctacagggtgtctaatcggttctccggcgtgcctgacaggttctccggctctggctccggcaccgatttcacactgaagatcagcagggtggaggctgaggacctgggcgtgtatttctgttttcagggcacccatgtgccatacacatttggctctggcaccaagctggagatcaag

SEQ ID NO: 54 - DNA, 336 bp, Artificial Sequence
  Nucleic acid sequence coding the light chain variable domain LA
gacgtggtcatgacacagagcccactgtctctgcctgtgaccctgggacagccagcctctatctcctgcaggtccagccagtccctggtgcacagctatggcaacacatacctgtattggtaccagcagaggcccggacagagcccaaggctgctgatctacagggtgtctaatcggttctccggcgtgcctgacaggtttagcggctctggctccggcaccgatttcacactgaagatctctagagtggaggctgaggatgtgggcgtgtatttctgttttcagggcacccatgtgccatacacatttggcggcggcaccaaggtggagatcaag

SEQ ID NO: 55 - DNA, 336 bp, Artificial Sequence
  Nucleic acid sequence coding the light chain variable domain LB
gacgtggtcatgacacagagcccactgtctctgcctgtgaccctgggacagccagcctctatctcctgcaggtccagccagtccctggtgcacagctacggcaacacatacctgtattggttccagcagaggcccggacagagcccaaggctgctgatctatagggtgtctaatcggttctccggcgtgcctgacaggtttagcggatctggatccggaaccgacttcaccctgaagatctctagagtggaggctgaggatgtgggcgtgtactattgtttccagggcacccatgtgccatacacatttggcggcggcaccaaggtggagatcaag

SEQ ID NO: 56 - protein, 456 aa, Mus musculus
QVQLQQPGAELVRPGSSVKLSCKASGYTFTSYWVHWVKQRPIQGLEWIGNIDPSDSDTHYNQKFKDKASLTVDKSSSTAYMQLSSLTFEDSAVYYCVRGGTGTMAWFAYWGQGTLVTVSAAKTTPPSVYPLAPGCGDTTGSSVTLGCLVKGYFPESVTVTWNSGSLSSSVHTFPALLQSGLYTMSSSVTVPSSTWPSQTVTCSVAHPASSTTVDKKLEPSGPISTINPCPPCKECHKCPAPNLEGGPSVFIFPPNIKDVLMISLTPKVTCVVVDVSEDDPDVQISWFVNNVEVHTAQTQTHREDYNSTIRVVSTLPIQHQDWMSGKEFKCKVNNKDLPSPIERTISKIKGLVRAPQVYILPPPAEQLSRKDVSLTCLVVGFNPGDISVEWTSNGHTEENYKDTAPVLDSDGSYFIYSKLNMKTSKWEKTDSFSCNVRHEGLKNYYLKKTISRSPGK

SEQ ID NO: 57 - protein, 219 aa, Mus musculus
DVVMTQTPLSLPVSLGDQASISCRSSQSLVHSYGNTYLYWYLQKPGQSPKLLIYRVSNRFSGVPDRFSGSGSGTDFTLKISRVEAEDLGVYFCFQGTHVPYTFGSGTKLEIKRADAAPTVSIFPPSSEQLTSGGASVVCFLNNFYPKDINVKWKIDGSERQNGVLNSWTDQDSKDSTYSMSSTLTLTKDEYERHNSYTCEATHKTSTSPIVKSFNRNEC

SEQ ID NO: 58 - DNA, 15 bp, Artificial Sequence
  Sequence coding HCDR1
agctattgggtgcac

SEQ ID NO: 59 - DNA, 15 bp, Artificial Sequence
  Sequence coding HCDR1
tcttattgggtgcac

SEQ ID NO: 60 - DNA, 15 bp, Artificial Sequence
  Sequence coding HCDR1
tcctattgggtgcac

SEQ ID NO: 61 - DNA, 51 bp, Artificial Sequence
  Sequence coding HCDR2
aacatcgaccccagcgactctgatacccattacaatcagaagtttaaggac

SEQ ID NO: 62 - DNA, 51 bp, Artificial Sequence
  Sequence coding HCDR2
aacatcgaccccagcgactctgatacacactactcccctagctttcagggc

SEQ ID NO: 63 - DNA, 33 bp, Artificial Sequence
  Sequence coding HCDR3
ggaggaaccggaacaatggcttggtttgcttac

SEQ ID NO: 64 - DNA, 33 bp, Artificial Sequence
  Sequence coding HCDR3
ggaggaaccggcacactggcttggttcgcttac

SEQ ID NO: 65 - DNA, 33 bp, Artificial Sequence
  Sequence coding HCDR3
ggaggaaccggaacaatggcttacttcgcttat

SEQ ID NO: 66 - DNA, 33 bp, Artificial Sequence
  Sequence coding HCDR3
ggaggaaccggcacactggcttacttcgcttat

SEQ ID NO: 67 - DNA, 48 bp, Artificial Sequence
  Sequence coding LCDR1
aggtccagccagtccctggtgcacagctatggcaacacatacctgtat

SEQ ID NO: 68 - DNA, 21 bp, Artificial Sequence
  Sequence coding LCDR2
agggtgtctaatcggttctcc

SEQ ID NO: 69 - DNA, 27 bp, Artificial Sequence
  Sequence coding LCDR3
tttcagggcacccatgtgccatacaca

SEQ ID NO: 70 - protein, 13 aa, Homo sapiens
ELIYNQKEGHFPR

SEQ ID NO: 71 - protein, 12 aa, Homo sapiens
RNNMDFSIRIGN

SEQ ID NO: 72 - protein, 9 aa, Homo sapiens
SPRDITLKW

SEQ ID NO: 73 - protein, 4 aa, Homo sapiens
YNQK